European Patent Application EP 4 527 933 A1, published March 26, 2025. Title: DUAL-VECTOR SYSTEM FOR TREATING HEARING IMPAIRMENT AND USE THEREOF. Applicant: SHANGHAI REFRESHGENE THERAPEUTICS CO., LTD. The sequence listing filed with the application follows.

SEQUENCE LISTING (9 sequences)

SEQ ID NO: 1 - protein, 1997 aa, homo sapiens
MALLIHLKTVSELRGRGDRIAKVTFRGQSFYSRVLENCEDVADFDETFRWPVASSIDRNEMLEIQVFNYSKVFSNKLIGTFRMVLQKVVEESHVEVTDTLIDDNNAIIKTSLCVEVRYQATDGTVGSWDDGDFLGDESLQEEEKDSQETDGLLPGSRPSSRPPGEKSFRRAGRSVFSAMKLGKNRSHKEEPQRPDEPAVLEMEDLDHLAIRLGDGLDPDSVSLASVTALTTNVSNKRSKPDIKMEPSAGRPMDYQVSITVIEARQLVGLNMDPVVCVEVGDDKKYTSMKESTNCPYYNEYFVFDFHVSPDVMFDKIIKISVIHSKNLLRSGTLVGSFKMDVGTVYSQPEHQFHHKWAILSDPDDISSGLKGYVKCDVAVVGKGDNIKTPHKANETDEDDIEGNLLLPEGVPPERQWARFYVKIYRAEGLPRMNTSLMANVKKAFIGENKDLVDPYVQVFFAGQKGKTSVQKSSYEPLWNEQVVFTDLFPPLCKRMKVQIRDSDKVNDVAIGTHFIDLRKISNDGDKGFLPTLGPAWVNMYGSTRNYTLLDEHQDLNEGLGEGVSFRARLLLGLAVEIVDTSNPELTSSTEVQVEQATPISESCAGKMEEFFLFGAFLEASMIDRRNGDKPITFEVTIGNYGNEVDGLSRPQRPRPRKEPGDEEEVDLIQNASDDEAGDAGDLASVSSTPPMRPQVTDRNYFHLPYLERKPCIYIKSWWPDQRRRLYNANIMDHIADKLEEGLNDIQEMIKTEKSYPERRLRGVLEELSCGCCRFLSLADKDQGHSSRTRLDRERLKSCMRELENMGQQARMLRAQVKRHTVRDKLRLCQNFLQKLRFLADEPQHSIPDIFIWMMSNNKRVAYARVPSKDLLFSIVEEETGKDCAKVKTLFLKLPGKRGFGSAGWTVQAKVELYLWLGLSKQRKEFLCGLPCGFQEVKAAQGLGLHAFPPVSLVYTKKQAFQLRAHMYQARSLFAADSSGLSDPFARVFFINQSQCTEVLNETLCPTWDQMLVFDNLELYGEAHELRDDPPIIVIEIYDQDSMGKADFMGRTFAKPLVKMADEAYCPPRFPPQLEYYQIYRGNATAGDLLAAFELLQIGPAGKADLPPINGPVDVDRGPIMPVPMGIRPVLSKYRVEVLFWGLRDLKRVNLAQVDRPRVDIECAGKGVQSSLIHNYKKNPNFNTLVKWFEVDLPENELLHPPLNIRVVDCRAFGRYTLVGSHAVSSLRRFIYRPPDRSAPSWNTTVRLLRRCRVLCNGGSSSHSTGEVVVTMEPEVPIKKLETMVKLDATSEAVVKVDVAEEEKEKKKKKKGTAEEPEEEEPDESMLDWWSKYFASIDTMKEQLRQQEPSGIDLEEKEEVDNTEGLKGSMKGKEKARAAKEEKKKKTQSSGSGQGSEAPEKKKPKIDELKVYPKELESEFDNFEDWLHTFNLLRGKTGDDEDGSTEEERIVGRFKGSLCVYKVPLPEDVSREAGYDSTYGMFQGIPSNDPINVLVRVYVVRATDLHPADINGKADPYIAIRLGKTDIRDKENYISKQLNPVFGKSFDIEASFPMESMLTVAVYDWDLVGTDDLIGETKIDLENRFYSKHRATCGIAQTYSTHGYNIWRDPMKPSQILTRLCKDGKVDGPHFGPPGRVKVANRVFTGPSEIEDENGQRKPTDEHVALLALRHWEDIPRAGCRLVPEHVETRPLLNPDKPGIEQGRLELWVDMFPMDMPAPGTPLDISPRKPKKYELRVIIWNTDEVVLEDDDFFTGEKSSDIFVRGWLKGQQEDKQDTDVHYHSLTGEGNFNWRYLFPFDYLAAEEKIVISKKESMFSWDETEYKIPARLTLQIWDADHFSADDFLGAIELDLNRFPRGAKTAKQCTMEMATGEVDVPLVSIFKQKRVKGWWPLLARNENDEFELTGKVEAELHLLTAEEAEKNPVGLARNEPDPLEKPNRPDTSFIWFLNPLKSARYFLWHTYRWLLLKLLLLLLLLLLLALFLYSVPGYLVKKILGA

SEQ ID NO: 2 - protein, 1997 aa, homo sapiens
MALLIHLKTVSELRGRGDRIAKVTFRGQSFYSRVLENCEDVADFDETFRWPVASSIDRNEMLEIQVFNYSKVFSNKLIGTFRMVLQKVVEESHVEVTDTLIDDNNAIIKTSLCVEVRYQATDGTVGSWDDGDFLGDESLQEEEKDSQETDGLLPGSRPSSRPPGEKSFRRAGRSVFSAMKLGKNRSHKEEPQRPDEPAVLEMEDLDHLAIRLGDGLDPDSVSLASVTALTTNVSNKRSKPDIKMEPSAGRPMDYQVSITVIEARQLVGLNMDPVVCVEVGDDKKYTSMKESTNCPYYNEYFVFDFHVSPDVMFDKIIKISVIHSKNLLRSGTLVGSFKMDVGTVYSQPEHQFHHKWAILSDPDDISSGLKGYVKCDVAVVGKGDNIKTPHKANETDEDDIEGNLLLPEGVPPERQWARFYVKIYRAEGLPRMNTSLMANVKKAFIGENKDLVDPYVQVFFAGQKGKTSVQKSSYEPLWNEQVVFTDLFPPLCKRMKVQIRDSDKVNDVAIGTHFIDLRKISNDGDKGFLPTLGPAWVNMYGSTRNYTLLDEHQDLNEGLGEGVSFRARLLLGLAVEIVDTSNPELTSSTEVQVEQATPISESCAGKMEEFFLFGAFLEASMIDRRNGDKPITFEVTIGNYGNEVDGLSRPQRPRPRKEPGDEEEVDLIQNASDDEAGDAGDLASVSSTPPMRPQVTDRNYFHLPYLERKPCIYIKSWWPDQRRRLYNANIMDHIADKLEEGLNDIQEMIKTEKSYPERRLRGVLEELSCGCCRFLSLADKDQGHSSRTRLDRERLKSCMRELENMGQQARMLRAQVKRHTVRDKLRLCQNFLQKLRFLADEPQHSIPDIFIWMMSNNKRVAYARVPSKDLLFSIVEEETGKDCAKVKTLFLKLPGKRGFGSAGWTVQAKVELYLWLGLSKQRKEFLCGLPCGFQEVKAAQGLGLHAFPPVSLVYTKKQAFQLRAHMYQARSLFAADSSGLSDPFARVFFINQSQCTEVLNETLCPTWDQMLVFDNLELYGEAHELRDDPPIIVIEIYDQDSMGKADFMGRTFAKPLVKMADEAYCPPRFPPQLEYYQIYRGNATAGDLLAAFELLQIGPAGKADLPPINGPVDVDRGPIMPVPMGIRPVLSKYRVEVLFWGLRDLKRVNLAQVDRPRVDIECAGKGVQSSLIHNYKKNPNFNTLVKWFEVDLPENELLHPPLNIRVVDCRAFGRYTLVGSHAVSSLRRFIYRPPDRSAPSWNTTVRLLRRCRVLCNGGSSSHSTGEVVVTMEPEVPIKKLETMVKLDATSEAVVKVDVAEEEKEKKKKKKGTAEEPEEEEPDESMLDWWSKYFASIDTMKEQLRQQEPSGIDLEEKEEVDNTEGLKGSMKGKEKARAAKEEKKKKTQSSGSGQGSEAPEKKKPKIDELKVYPKELESEFDNFEDWLHTFNLLRGKTGDDEDGSTEEERIVGRFKGSLCVYKVPLPEDVSREAGYDSTYGMFQGIPSNDPINVLVRVYVVRATDLHPADINGKADPYIAIRLGKTDIRDKENYISKQLNPVFGKSFDIEASFPMESMLTVAVYDWDLVGTDDLIGETKIDLENRFYSKHRATCGIAQTYSTHGYNIWRDPMKPSQILTRLCKDGKVDGPHFGPPGRVKVANRVFTGPSEIEDENGQRKPTDEHVALLALRHWEDIPRAGCRLVPEHVETRPLLNPDKPGIEQGRLELWVDMFPMDMPAPGTPLDISPRKPKKYELRVIIWNTDEVVLEDDDFFTGEKSSDIFVRGWLKGQQEDKQDTDVHYHSLTGEGNFNWRYLFPFDYLAAEEKIVISKKESMFSWDETEYKIPARLTLQIWDADHFSADDFLGAIELDLNRFPRGAKTAKQCTMEMATGEVDVPLVSIFKQKRVKGWWPLLARNENDEFELTGKVEAELHLLTAEEAEKNPVGLARNEPDPLEKPNRPDTAFVWFLNPLKSIKYLICTRYKWLIIKIVLALLGLLMLGLFLYSLPGYMVKKLLGA

SEQ ID NO: 3 - DNA, 5994 bp, homo sapiens
  source 1..5994: mol_type = other DNA
atggccttgctcatccacctcaagacagtctcggagctgcggggcaggggcgaccggatcgccaaagtgactttccgagggcaatccttctactctcgggtcctggagaactgtgaggatgtggctgactttgatgagacatttcggtggccggtggccagcagcatcgacagaaatgagatgctggagattcaggttttcaactacagcaaagtcttcagcaacaagctcatcgggaccttccgcatggtgctgcagaaggtggtagaggagagccatgtggaggtgactgacacgctgattgatgacaacaatgctatcatcaagaccagcctgtgcgtggaggtccggtatcaggccactgacggcacagtgggctcctgggacgatggggacttcctgggagatgagtctcttcaagaggaagagaaggacagccaagagacggatggactgctcccaggctcccggcccagctcccggcccccaggagagaagagcttccggagagccgggaggagcgtgttctccgccatgaagctcggcaaaaaccggtctcacaaggaggagccccaaagaccagatgaaccggcggtgctggagatggaagaccttgaccatctggccattcggctaggagatggactggatcccgactcggtgtctctagcctcagtcacagctctcaccactaatgtctccaacaagcgatctaagccagacattaagatggagccaagtgctgggcggcccatggattaccaggtcagcatcacggtgatcgaggcccggcagctggtgggcttgaacatggaccctgtggtgtgcgtggaggtgggtgacgacaagaagtacacatccatgaaggagtccactaactgcccctattacaacgagtacttcgtcttcgacttccatgtctctccggatgtcatgtttgacaagatcatcaagatttcggtgattcactccaagaacctgctgcgcagtggcaccctggtgggctccttcaaaatggacgtgggaaccgtgtactcgcagccagagcaccagttccatcacaagtgggccatcctgtctgaccccgatgacatctcctcggggctgaagggctacgtgaagtgtgacgttgccgtggtgggcaaaggggacaacatcaagacgccccacaaggccaatgagaccgacgaagatgacattgaggggaacttgctgctccccgagggggtgccccccgaacgccagtgggcccggttctatgtgaaaatttaccgagcagaggggctgccccgtatgaacacaagcctcatggccaatgtaaagaaggctttcatcggtgaaaacaaggacctcgtggacccctacgtgcaagtcttctttgctggccagaagggcaagacttcagtgcagaagagcagctatgagcccctgtggaatgagcaggtcgtctttacagacctcttccccccactctgcaaacgcatgaaggtgcagatccgagactcggacaaggtcaacgacgtggccatcggcacccacttcattgacctgcgcaagatttctaatgacggagacaaaggcttcctgcccacactgggcccagcctgggtgaacatgtacggctccacacgtaactacacgctgctggatgagcatcaggacctgaacgagggcctgggggagggtgtgtccttccgggcccggctcctgctgggcctggctgtggagatcgtagacacctccaaccctgagctcaccagctccacagaggtgcaggtggagcaggccacgcccatctcggagagctgtgcaggtaaaatggaagaattctttctctttggagccttcctggaggcctcaatgatcgaccggagaaacggagacaagcccatcacctttgaggtcaccataggcaactatgggaacgaagttgatggcctgtcccggccccagcggcctcggccccggaaggagccgggggatgaggaagaagtagacctgattcagaacgcaagtgatgacgaggccggtgatgccggggacctggcctcagtctcctccactccaccaatgcggccccaggtcaccgacaggaactacttccatctgccctacctggagcgaaagccctgcatctacatcaagagctggtggccggaccagcgccgccgcctctacaatgccaacatcatggaccacattgccgacaagctggaagaaggcctgaacgacatacaggagatgatcaaaacggagaagtcctaccctgagcgtcgcctgcggggcgtcctggaggagctgagctgtggctgctgccgcttcctctccctcgctgacaaggaccagggccactcatcccgcaccaggcttgaccgggagcgcctcaagtcctgcatgagggagctggaaaacatggggcagcaggccaggatgctgcgggcccaggtgaagcggcacacggtgcgggacaagctgaggctgtgccagaacttcctgcagaagctgcgcttcctggcggacgagccccagcacagcattcccgacatcttcatctggatgatgagcaacaacaagcgtgtcgcctatgcccgtgtgccctccaaggacctgctcttctccatcgtggaggaggagactggcaaggactgcgccaaggtcaagacgctcttccttaagctgccagggaagcggggcttcggctcggcaggctggacagtgcaggccaaggtggagctgtacctgtggctgggcctcagcaaacagcgcaaggagttcctgtgcggcctgccctgtggcttccaggaggtcaaggcagcccagggcctgggcctgcatgccttcccacccgtcagcctggtctacaccaagaagcaggcgttccagctccgagcgcacatgtaccaggcccgcagcctctttgccgccgacagcagcggactctcagacccctttgcccgcgtcttcttcatcaatcagagtcagtgcacagaggtgctgaatgagaccctgtgtcccacctgggaccagatgctggtgttcgacaacctggagctctatggtgaagctcatgagctgagggacgatccgcccatcattgtcattgaaatctatgaccaggattccatgggcaaagctgacttcatgggccggaccttcgccaaacccctggtgaagatggcagacgaggcgtactgcccaccccgcttcccacctcagctcgagtactaccagatctaccgtggcaacgccacagctggagacctgctggcggccttcgagctgctgcagattggaccagcagggaaggctgacctgccccccatcaatggcccggtggacgtggaccgaggtcccatcatgcccgtgcccatgggcatccggcccgtgctcagcaagtaccgagtggaggtgctgttctggggcctacgggacctaaagcgggtgaacctggcccaggtggaccggccacgggtggacatcgagtgtgcagggaagggggtgcagtcgtccctgatccacaattataagaagaaccccaacttcaacaccctcgtcaagtggtttgaagtggacctcccagagaacgagctgctgcacccgcccttgaacatccgtgtggtggactgccgggccttcggtcgctacacactggtgggctcccatgccgtcagctccctgcgacgcttcatctaccggcccccagaccgctcggcccccagctggaacaccacggtcaggcttctccggcgctgccgtgtgctgtgcaatgggggctcctcctctcactccacaggggaggttgtggtgactatggagccagaggtacccatcaagaaactggagaccatggtgaagctggacgcgacttctgaagctgttgtcaaggtggatgtggctgaggaggagaaggagaagaagaagaagaagaagggcactgcggaggagccagaggaggaggagccagacgagagcatgctggactggtggtccaagtactttgcctccattgacaccatgaaggagcaacttcgacaacaagagccctctggaattgacttggaggagaaggaggaagtggacaataccgagggcctgaaggggtcaatgaagggcaaggagaaggcaagggctgccaaagaggagaagaagaagaaaactcagagctctggctctggccaggggtccgaggcccccgagaagaagaaacccaagattgatgagcttaaggtataccccaaagagctggagtccgagtttgataactttgaggactggctgcacactttcaacttgcttcggggcaagaccggggatgatgaggatggctccaccgaggaggagcgcattgtgggacgcttcaagggctccctctgcgtgtacaaagtgccactcccagaggacgtgtcccgggaagccggctacgactccacctacggcatgttccagggcatcccgagcaatgaccccatcaatgtgctggtccgagtctatgtggtccgggccacggacctgcaccctgctgacatcaacggcaaagctgacccctacatcgccatccggctaggcaagactgacatccgcgacaaggagaactacatctccaagcagctcaaccctgtctttgggaagtcctttgacatcgaggcctccttccccatggaatccatgctgacggtggctgtgtatgactgggacctggtgggcactgatgacctcattggggaaaccaagatcgacctggagaaccgcttctacagcaagcaccgcgccacctgcggcatcgcccagacctactccacacatggctacaatatctggcgggaccccatgaagcccagccagatcctgacccgcctctgcaaagacggcaaagtggacggcccccactttgggccccctgggagagtgaaggtggccaaccgcgtcttcactgggccctctgagattgaggacgagaacggtcagaggaagcccacagacgagcatgtggcgctgttggccctgaggcactgggaggacatcccccgcgcaggctgccgcctggtgccagagcatgtggagacgaggccgctgctcaaccccgacaagccgggcatcgagcagggccgcctggagctgtgggtggacatgttccccatggacatgccagcccctgggacgcctctggacatctcacctcggaagcccaagaagtacgagctgcgggtcatcatctggaacacagatgaggtggtcttggaggacgacgacttcttcacaggggagaagtccagtgacatcttcgtgagggggtggctgaagggccagcaggaggacaagcaggacacagacgtccactaccactccctcactggcgagggcaacttcaactggcgctacctgttccccttcgactacctggcggcggaggagaagatcgtcatctccaagaaggagtccatgttctcctgggacgagaccgagtacaagatccccgcgcggctcaccctgcagatctgggatgcggaccacttctccgctgacgacttcctgggggccatcgagctggacctgaaccggttcccgcggggcgcaaagacagccaagcagtgcaccatggagatggccaccggggaggtggacgtgcccctcgtgtccatcttcaagcaaaagcgcgtcaaaggctggtggcccctcctggcccgcaatgagaacgatgagtttgagctcacgggcaaggtggaggctgagctgcatttactgacagcagaggaggcagagaagaacccagtgggcctggcccgcaatgaacctgaccccctagagaaacccaaccggcccgacacgagcttcatctggttcctgaaccctctcaagtcggctcgctacttcttgtggcacacgtatcgctggctgctcctcaaactgttgctgctcctgctgctgctcctcctcctcgccctgttcctctactctgtgcctggctacctggtcaagaaaatcctcggggcctga

SEQ ID NO: 4 - DNA, 5994 bp, homo sapiens
  source 1..5994: mol_type = other DNA
atggccttgctcatccacctcaagacagtctcggagctgcggggcaggggcgaccggatcgccaaagtgactttccgagggcaatccttctactctcgggtcctggagaactgtgaggatgtggctgactttgatgagacatttcggtggccggtggccagcagcatcgacagaaatgagatgctggagattcaggttttcaactacagcaaagtcttcagcaacaagctcatcgggaccttccgcatggtgctgcagaaggtggtagaggagagccatgtggaggtgactgacacgctgattgatgacaacaatgctatcatcaagaccagcctgtgcgtggaggtccggtatcaggccactgacggcacagtgggctcctgggacgatggggacttcctgggagatgagtctcttcaagaggaagagaaggacagccaagagacggatggactgctcccaggctcccggcccagctcccggcccccaggagagaagagcttccggagagccgggaggagcgtgttctccgccatgaagctcggcaaaaaccggtctcacaaggaggagccccaaagaccagatgaaccggcggtgctggagatggaagaccttgaccatctggccattcggctaggagatggactggatcccgactcggtgtctctagcctcagtcacagctctcaccactaatgtctccaacaagcgatctaagccagacattaagatggagccaagtgctgggcggcccatggattaccaggtcagcatcacggtgatcgaggcccggcagctggtgggcttgaacatggaccctgtggtgtgcgtggaggtgggtgacgacaagaagtacacatccatgaaggagtccactaactgcccctattacaacgagtacttcgtcttcgacttccatgtctctccggatgtcatgtttgacaagatcatcaagatttcggtgattcactccaagaacctgctgcgcagtggcaccctggtgggctccttcaaaatggacgtgggaaccgtgtactcgcagccagagcaccagttccatcacaagtgggccatcctgtctgaccccgatgacatctcctcggggctgaagggctacgtgaagtgtgacgttgccgtggtgggcaaaggggacaacatcaagacgccccacaaggccaatgagaccgacgaagatgacattgaggggaacttgctgctccccgagggggtgccccccgaacgccagtgggcccggttctatgtgaaaatttaccgagcagaggggctgccccgtatgaacacaagcctcatggccaatgtaaagaaggctttcatcggtgaaaacaaggacctcgtggacccctacgtgcaagtcttctttgctggccagaagggcaagacttcagtgcagaagagcagctatgagcccctgtggaatgagcaggtcgtctttacagacctcttccccccactctgcaaacgcatgaaggtgcagatccgagactcggacaaggtcaacgacgtggccatcggcacccacttcattgacctgcgcaagatttctaatgacggagacaaaggcttcctgcccacactgggcccagcctgggtgaacatgtacggctccacacgtaactacacgctgctggatgagcatcaggacctgaacgagggcctgggggagggtgtgtccttccgggcccggctcctgctgggcctggctgtggagatcgtagacacctccaaccctgagctcaccagctccacagaggtgcaggtggagcaggccacgcccatctcggagagctgtgcaggtaaaatggaagaattctttctctttggagccttcctggaggcctcaatgatcgaccggagaaacggagacaagcccatcacctttgaggtcaccataggcaactatgggaacgaagttgatggcctgtcccggccccagcggcctcggccccggaaggagccgggggatgaggaagaagtagacctgattcagaacgcaagtgatgacgaggccggtgatgccggggacctggcctcagtctcctccactccaccaatgcggccccaggtcaccgacaggaactacttccatctgccctacctggagcgaaagccctgcatctacatcaagagctggtggccggaccagcgccgccgcctctacaatgccaacatcatggaccacattgccgacaagctggaagaaggcctgaacgacatacaggagatgatcaaaacggagaagtcctaccctgagcgtcgcctgcggggcgtcctggaggagctgagctgtggctgctgccgcttcctctccctcgctgacaaggaccagggccactcatcccgcaccaggcttgaccgggagcgcctcaagtcctgcatgagggagctggaaaacatggggcagcaggccaggatgctgcgggcccaggtgaagcggcacacggtgcgggacaagctgaggctgtgccagaacttcctgcagaagctgcgcttcctggcggacgagccccagcacagcattcccgacatcttcatctggatgatgagcaacaacaagcgtgtcgcctatgcccgtgtgccctccaaggacctgctcttctccatcgtggaggaggagactggcaaggactgcgccaaggtcaagacgctcttccttaagctgccagggaagcggggcttcggctcggcaggctggacagtgcaggccaaggtggagctgtacctgtggctgggcctcagcaaacagcgcaaggagttcctgtgcggcctgccctgtggcttccaggaggtcaaggcagcccagggcctgggcctgcatgccttcccacccgtcagcctggtctacaccaagaagcaggcgttccagctccgagcgcacatgtaccaggcccgcagcctctttgccgccgacagcagcggactctcagacccctttgcccgcgtcttcttcatcaatcagagtcagtgcacagaggtgctgaatgagaccctgtgtcccacctgggaccagatgctggtgttcgacaacctggagctctatggtgaagctcatgagctgagggacgatccgcccatcattgtcattgaaatctatgaccaggattccatgggcaaagctgacttcatgggccggaccttcgccaaacccctggtgaagatggcagacgaggcgtactgcccaccccgcttcccacctcagctcgagtactaccagatctaccgtggcaacgccacagctggagacctgctggcggccttcgagctgctgcagattggaccagcagggaaggctgacctgccccccatcaatggcccggtggacgtggaccgaggtcccatcatgcccgtgcccatgggcatccggcccgtgctcagcaagtaccgagtggaggtgctgttctggggcctacgggacctaaagcgggtgaacctggcccaggtggaccggccacgggtggacatcgagtgtgcagggaagggggtgcagtcgtccctgatccacaattataagaagaaccccaacttcaacaccctcgtcaagtggtttgaagtggacctcccagagaacgagctgctgcacccgcccttgaacatccgtgtggtggactgccgggccttcggtcgctacacactggtgggctcccatgccgtcagctccctgcgacgcttcatctaccggcccccagaccgctcggcccccagctggaacaccacggtcaggcttctccggcgctgccgtgtgctgtgcaatgggggctcctcctctcactccacaggggaggttgtggtgactatggagccagaggtacccatcaagaaactggagaccatggtgaagctggacgcgacttctgaagctgttgtcaaggtggatgtggctgaggaggagaaggagaagaagaagaagaagaagggcactgcggaggagccagaggaggaggagccagacgagagcatgctggactggtggtccaagtactttgcctccattgacaccatgaaggagcaacttcgacaacaagagccctctggaattgacttggaggagaaggaggaagtggacaataccgagggcctgaaggggtcaatgaagggcaaggagaaggcaagggctgccaaagaggagaagaagaagaaaactcagagctctggctctggccaggggtccgaggcccccgagaagaagaaacccaagattgatgagcttaaggtataccccaaagagctggagtccgagtttgataactttgaggactggctgcacactttcaacttgcttcggggcaagaccggggatgatgaggatggctccaccgaggaggagcgcattgtgggacgcttcaagggctccctctgcgtgtacaaagtgccactcccagaggacgtgtcccgggaagccggctacgactccacctacggcatgttccagggcatcccgagcaatgaccccatcaatgtgctggtccgagtctatgtggtccgggccacggacctgcaccctgctgacatcaacggcaaagctgacccctacatcgccatccggctaggcaagactgacatccgcgacaaggagaactacatctccaagcagctcaaccctgtctttgggaagtcctttgacatcgaggcctccttccccatggaatccatgctgacggtggctgtgtatgactgggacctggtgggcactgatgacctcattggggaaaccaagatcgacctggagaaccgcttctacagcaagcaccgcgccacctgcggcatcgcccagacctactccacacatggctacaatatctggcgggaccccatgaagcccagccagatcctgacccgcctctgcaaagacggcaaagtggacggcccccactttgggccccctgggagagtgaaggtggccaaccgcgtcttcactgggccctctgagattgaggacgagaacggtcagaggaagcccacagacgagcatgtggcgctgttggccctgaggcactgggaggacatcccccgcgcaggctgccgcctggtgccagagcatgtggagacgaggccgctgctcaaccccgacaagccgggcatcgagcagggccgcctggagctgtgggtggacatgttccccatggacatgccagcccctgggacgcctctggacatctcacctcggaagcccaagaagtacgagctgcgggtcatcatctggaacacagatgaggtggtcttggaggacgacgacttcttcacaggggagaagtccagtgacatcttcgtgagggggtggctgaagggccagcaggaggacaagcaggacacagacgtccactaccactccctcactggcgagggcaacttcaactggcgctacctgttccccttcgactacctggcggcggaggagaagatcgtcatctccaagaaggagtccatgttctcctgggacgagaccgagtacaagatccccgcgcggctcaccctgcagatctgggatgcggaccacttctccgctgacgacttcctgggggccatcgagctggacctgaaccggttcccgcggggcgcaaagacagccaagcagtgcaccatggagatggccaccggggaggtggacgtgcccctcgtgtccatcttcaagcaaaagcgcgtcaaaggctggtggcccctcctggcccgcaatgagaacgatgagtttgagctcacgggcaaggtggaggctgagctgcatttactgacagcagaggaggcagagaagaacccagtgggcctggcccgcaatgaacctgaccccctagagaaacccaaccggcccgacacggccttcgtctggttcctcaaccctctcaagtccatcaagtacctcatctgcacccggtacaagtggctcatcatcaagatcgtgctggcgctgttggggctgctcatgttggggctcttcctctacagcctccctggctacatggtcaaaaagctccttggggcatga

SEQ ID NO: 5 - DNA, 2844 bp, synthetic construct
  source 1..2844: mol_type = other DNA
ggattcgaacatcgattgaattccccggggatcctctaggccaccatggccttgctcatccacctcaagacagtctcggagctgcggggcaggggcgaccggatcgccaaagtgactttccgagggcaatccttctactctcgggtcctggagaactgtgaggatgtggctgactttgatgagacatttcggtggccggtggccagcagcatcgacagaaatgagatgctggagattcaggttttcaactacagcaaagtcttcagcaacaagctcatcgggaccttccgcatggtgctgcagaaggtggtagaggagagccatgtggaggtgactgacacgctgattgatgacaacaatgctatcatcaagaccagcctgtgcgtggaggtccggtatcaggccactgacggcacagtgggctcctgggacgatggggacttcctgggagatgagtctcttcaagaggaagagaaggacagccaagagacggatggactgctcccaggctcccggcccagctcccggcccccaggagagaagagcttccggagagccgggaggagcgtgttctccgccatgaagctcggcaaaaaccggtctcacaaggaggagccccaaagaccagatgaaccggcggtgctggagatggaagaccttgaccatctggccattcggctaggagatggactggatcccgactcggtgtctctagcctcagtcacagctctcaccactaatgtctccaacaagcgatctaagccagacattaagatggagccaagtgctgggcggcccatggattaccaggtcagcatcacggtgatcgaggcccggcagctggtgggcttgaacatggaccctgtggtgtgcgtggaggtgggtgacgacaagaagtacacatccatgaaggagtccactaactgcccctattacaacgagtacttcgtcttcgacttccatgtctctccggatgtcatgtttgacaagatcatcaagatttcggtgattcactccaagaacctgctgcgcagtggcaccctggtgggctccttcaaaatggacgtgggaaccgtgtactcgcagccagagcaccagttccatcacaagtgggccatcctgtctgaccccgatgacatctcctcggggctgaagggctacgtgaagtgtgacgttgccgtggtgggcaaaggggacaacatcaagacgccccacaaggccaatgagaccgacgaagatgacattgaggggaacttgctgctccccgagggggtgccccccgaacgccagtgggcccggttctatgtgaaaatttaccgagcagaggggctgccccgtatgaacacaagcctcatggccaatgtaaagaaggctttcatcggtgaaaacaaggacctcgtggacccctacgtgcaagtcttctttgctggccagaagggcaagacttcagtgcagaagagcagctatgagcccctgtggaatgagcaggtcgtctttacagacctcttccccccactctgcaaacgcatgaaggtgcagatccgagactcggacaaggtcaacgacgtggccatcggcacccacttcattgacctgcgcaagatttctaatgacggagacaaaggcttcctgcccacactgggcccagcctgggtgaacatgtacggctccacacgtaactacacgctgctggatgagcatcaggacctgaacgagggcctgggggagggtgtgtccttccgggcccggctcctgctgggcctggctgtggagatcgtagacacctccaaccctgagctcaccagctccacagaggtgcaggtggagcaggccacgcccatctcggagagctgtgcaggtaaaatggaagaattctttctctttggagccttcctggaggcctcaatgatcgaccggagaaacggagacaagcccatcacctttgaggtcaccataggcaactatgggaacgaagttgatggcctgtcccggccccagcggcctcggccccggaaggagccgggggatgaggaagaagtagacctgattcagaacgcaagtgatgacgaggccggtgatgccggggacctggcctcagtctcctccactccaccaatgcggccccaggtcaccgacaggaactacttccatctgccctacctggagcgaaagccctgcatctacatcaagagctggtggccggaccagcgccgccgcctctacaatgccaacatcatggaccacattgccgacaagctggaagaaggcctgaacgacatacaggagatgatcaaaacggagaagtcctaccctgagcgtcgcctgcggggcgtcctggaggagctgagctgtggctgctgccgcttcctctccctcgctgacaaggaccagggccactcatcccgcaccaggcttgaccgggagcgcctcaagtcctgcatgagggagctggaaaacatggggcagcaggccaggatgctgcgggcccaggtgaagcggcacacggtgcgggacaagctgaggctgtgtctggctggcgatactctcattaccctggccgatggacgacgagtgcctattagagaactggtgtcacagcagaatttttccgtgtgggctctgaatcctcagacttaccgcctggagagggctagagtgagtagagctttctgtaccggcatcaaacctgtgtaccgcctcaccactagactggggagatccattagggccactgccaaccaccgatttctcacacctcagggctggaaacgagtcgatgaactccagcctggagattacctggctctgcctaggagaatccctactgcctcctaaaagcttgcc

SEQ ID NO: 6 - DNA, 3723 bp, synthetic construct
  source 1..3723: mol_type = other DNA
ggattcgaacatcgattgaattccccggggatcctctaggccaccatggcggcggcgtgcccggaactgcgtcagctggcgcagagcgatgtgtattgggatccgattgtgagcattgaaccggatggcgtggaagaagtgtttgatctgaccgtgccgggcccgcataactttgtggcgaacgatattattgcgcataactgccagaacttcctgcagaagctgcgcttcctggcggacgagccccagcacagcattcccgacatcttcatctggatgatgagcaacaacaagcgtgtcgcctatgcccgtgtgccctccaaggacctgctcttctccatcgtggaggaggagactggcaaggactgcgccaaggtcaagacgctcttccttaagctgccagggaagcggggcttcggctcggcaggctggacagtgcaggccaaggtggagctgtacctgtggctgggcctcagcaaacagcgcaaggagttcctgtgcggcctgccctgtggcttccaggaggtcaaggcagcccagggcctgggcctgcatgccttcccacccgtcagcctggtctacaccaagaagcaggcgttccagctccgagcgcacatgtaccaggcccgcagcctctttgccgccgacagcagcggactctcagacccctttgcccgcgtcttcttcatcaatcagagtcagtgcacagaggtgctgaatgagaccctgtgtcccacctgggaccagatgctggtgttcgacaacctggagctctatggtgaagctcatgagctgagggacgatccgcccatcattgtcattgaaatctatgaccaggattccatgggcaaagctgacttcatgggccggaccttcgccaaacccctggtgaagatggcagacgaggcgtactgcccaccccgcttcccacctcagctcgagtactaccagatctaccgtggcaacgccacagctggagacctgctggcggccttcgagctgctgcagattggaccagcagggaaggctgacctgccccccatcaatggcccggtggacgtggaccgaggtcccatcatgcccgtgcccatgggcatccggcccgtgctcagcaagtaccgagtggaggtgctgttctggggcctacgggacctaaagcgggtgaacctggcccaggtggaccggccacgggtggacatcgagtgtgcagggaagggggtgcagtcgtccctgatccacaattataagaagaaccccaacttcaacaccctcgtcaagtggtttgaagtggacctcccagagaacgagctgctgcacccgcccttgaacatccgtgtggtggactgccgggccttcggtcgctacacactggtgggctcccatgccgtcagctccctgcgacgcttcatctaccggcccccagaccgctcggcccccagctggaacaccacggtcaggcttctccggcgctgccgtgtgctgtgcaatgggggctcctcctctcactccacaggggaggttgtggtgactatggagccagaggtacccatcaagaaactggagaccatggtgaagctggacgcgacttctgaagctgttgtcaaggtggatgtggctgaggaggagaaggagaagaagaagaagaagaagggcactgcggaggagccagaggaggaggagccagacgagagcatgctggactggtggtccaagtactttgcctccattgacaccatgaaggagcaacttcgacaacaagagccctctggaattgacttggaggagaaggaggaagtggacaataccgagggcctgaaggggtcaatgaagggcaaggagaaggcaagggctgccaaagaggagaagaagaagaaaactcagagctctggctctggccaggggtccgaggcccccgagaagaagaaacccaagattgatgagcttaaggtataccccaaagagctggagtccgagtttgataactttgaggactggctgcacactttcaacttgcttcggggcaagaccggggatgatgaggatggctccaccgaggaggagcgcattgtgggacgcttcaagggctccctctgcgtgtacaaagtgccactcccagaggacgtgtcccgggaagccggctacgactccacctacggcatgttccagggcatcccgagcaatgaccccatcaatgtgctggtccgagtctatgtggtccgggccacggacctgcaccctgctgacatcaacggcaaagctgacccctacatcgccatccggctaggcaagactgacatccgcgacaaggagaactacatctccaagcagctcaaccctgtctttgggaagtcctttgacatcgaggcctccttccccatggaatccatgctgacggtggctgtgtatgactgggacctggtgggcactgatgacctcattggggaaaccaagatcgacctggagaaccgcttctacagcaagcaccgcgccacctgcggcatcgcccagacctactccacacatggctacaatatctggcgggaccccatgaagcccagccagatcctgacccgcctctgcaaagacggcaaagtggacggcccccactttgggccccctgggagagtgaaggtggccaaccgcgtcttcactgggccctctgagattgaggacgagaacggtcagaggaagcccacagacgagcatgtggcgctgttggccctgaggcactgggaggacatcccccgcgcaggctgccgcctggtgccagagcatgtggagacgaggccgctgctcaaccccgacaagccgggcatcgagcagggccgcctggagctgtgggtggacatgttccccatggacatgccagcccctgggacgcctctggacatctcacctcggaagcccaagaagtacgagctgcgggtcatcatctggaacacagatgaggtggtcttggaggacgacgacttcttcacaggggagaagtccagtgacatcttcgtgagggggtggctgaagggccagcaggaggacaagcaggacacagacgtccactaccactccctcactggcgagggcaacttcaactggcgctacctgttccccttcgactacctggcggcggaggagaagatcgtcatctccaagaaggagtccatgttctcctgggacgagaccgagtacaagatccccgcgcggctcaccctgcagatctgggatgcggaccacttctccgctgacgacttcctgggggccatcgagctggacctgaaccggttcccgcggggcgcaaagacagccaagcagtgcaccatggagatggccaccggggaggtggacgtgcccctcgtgtccatcttcaagcaaaagcgcgtcaaaggctggtggcccctcctggcccgcaatgagaacgatgagtttgagctcacgggcaaggtggaggctgagctgcatttactgacagcagaggaggcagagaagaacccagtgggcctggcccgcaatgaacctgaccccctagagaaacccaaccggcccgacacggccttcgtctggttcctcaaccctctcaagtccatcaagtacctcatctgcacccggtacaagtggctcatcatcaagatcgtgctggcgctgttggggctgctcatgttggggctcttcctctacagcctccctggctacatggtcaaaaagctccttggggcatgaaagcttgcc

SEQ ID NO: 7 - DNA, 3153 bp, synthetic construct
  source 1..3153: mol_type = other DNA
ggattcgaacatcgattgaattccccggggatcctctaggccaccatggccttgctcatccacctcaagacagtctcggagctgcggggcaggggcgaccggatcgccaaagtgactttccgagggcaatccttctactctcgggtcctggagaactgtgaggatgtggctgactttgatgagacatttcggtggccggtggccagcagcatcgacagaaatgagatgctggagattcaggttttcaactacagcaaagtcttcagcaacaagctcatcgggaccttccgcatggtgctgcagaaggtggtagaggagagccatgtggaggtgactgacacgctgattgatgacaacaatgctatcatcaagaccagcctgtgcgtggaggtccggtatcaggccactgacggcacagtgggctcctgggacgatggggacttcctgggagatgagtctcttcaagaggaagagaaggacagccaagagacggatggactgctcccaggctcccggcccagctcccggcccccaggagagaagagcttccggagagccgggaggagcgtgttctccgccatgaagctcggcaaaaaccggtctcacaaggaggagccccaaagaccagatgaaccggcggtgctggagatggaagaccttgaccatctggccattcggctaggagatggactggatcccgactcggtgtctctagcctcagtcacagctctcaccactaatgtctccaacaagcgatctaagccagacattaagatggagccaagtgctgggcggcccatggattaccaggtcagcatcacggtgatcgaggcccggcagctggtgggcttgaacatggaccctgtggtgtgcgtggaggtgggtgacgacaagaagtacacatccatgaaggagtccactaactgcccctattacaacgagtacttcgtcttcgacttccatgtctctccggatgtcatgtttgacaagatcatcaagatttcggtgattcactccaagaacctgctgcgcagtggcaccctggtgggctccttcaaaatggacgtgggaaccgtgtactcgcagccagagcaccagttccatcacaagtgggccatcctgtctgaccccgatgacatctcctcggggctgaagggctacgtgaagtgtgacgttgccgtggtgggcaaaggggacaacatcaagacgccccacaaggccaatgagaccgacgaagatgacattgaggggaacttgctgctccccgagggggtgccccccgaacgccagtgggcccggttctatgtgaaaatttaccgagcagaggggctgccccgtatgaacacaagcctcatggccaatgtaaagaaggctttcatcggtgaaaacaaggacctcgtggacccctacgtgcaagtcttctttgctggccagaagggcaagacttcagtgcagaagagcagctatgagcccctgtggaatgagcaggtcgtctttacagacctcttccccccactctgcaaacgcatgaaggtgcagatccgagactcggacaaggtcaacgacgtggccatcggcacccacttcattgacctgcgcaagatttctaatgacggagacaaaggcttcctgcccacactgggcccagcctgggtgaacatgtacggctccacacgtaactacacgctgctggatgagcatcaggacctgaacgagggcctgggggagggtgtgtccttccgggcccggctcctgctgggcctggctgtggagatcgtagacacctccaaccctgagctcaccagctccacagaggtgcaggtggagcaggccacgcccatctcggagagctgtgcaggtaaaatggaagaattctttctctttggagccttcctggaggcctcaatgatcgaccggagaaacggagacaagcccatcacctttgaggtcaccataggcaactatgggaacgaagttgatggcctgtcccggccccagcggcctcggccccggaaggagccgggggatgaggaagaagtagacctgattcagaacgcaagtgatgacgaggccggtgatgccggggacctggcctcagtctcctccactccaccaatgcggccccaggtcaccgacaggaactacttccatctgccctacctggagcgaaagccctgcatctacatcaagagctggtggccggaccagcgccgccgcctctacaatgccaacatcatggaccacattgccgacaagctggaagaaggcctgaacgacatacaggagatgatcaaaacggagaagtcctaccctgagcgtcgcctgcggggcgtcctggaggagctgagctgtggctgctgccgcttcctctccctcgctgacaaggaccagggccactcatcccgcaccaggcttgaccgggagcgcctcaagtcctgcatgagggagctggaaaacatggggcagcaggccaggatgctgcgggcccaggtgaagcggcacacggtgcgggacaagctgaggctgtgccagaacttcctgcagaagctgcgcttcctggcggacgagccccagcacagcattcccgacatcttcatctggatgatgagcaacaacaagcgtgtcgcctatgcccgtgtgccctccaaggacctgctcttctccatcgtggaggaggagactggcaaggactgcgccaaggtcaagacgctcttccttaagctgccagggaagcggggcttcggctcggcaggctggacagtgcaggccaaggtggagctgtacctgtggctgggcctcagcaaacagcgcaaggagttcctgtgcggcctgccctgtctggctggcgatactctcattaccctggccgatggacgacgagtgcctattagagaactggtgtcacagcagaatttttccgtgtgggctctgaatcctcagacttaccgcctggagagggctagagtgagtagagctttctgtaccggcatcaaacctgtgtaccgcctcaccactagactggggagatccattagggccactgccaaccaccgatttctcacacctcagggctggaaacgagtcgatgaactccagcctggagattacctggctctgcctaggagaatccctactgcctcctaaaagcttgcc

SEQ ID NO: 8 - DNA, 3414 bp, synthetic construct
  source 1..3414: mol_type = other DNA
ggattcgaacatcgattgaattccccggggatcctctaggccaccatggcggcggcgtgcccggaactgcgtcagctggcgcagagcgatgtgtattgggatccgattgtgagcattgaaccggatggcgtggaagaagtgtttgatctgaccgtgccgggcccgcataactttgtggcgaacgatattattgcgcataactgtggcttccaggaggtcaaggcagcccagggcctgggcctgcatgccttcccacccgtcagcctggtctacaccaagaagcaggcgttccagctccgagcgcacatgtaccaggcccgcagcctctttgccgccgacagcagcggactctcagacccctttgcccgcgtcttcttcatcaatcagagtcagtgcacagaggtgctgaatgagaccctgtgtcccacctgggaccagatgctggtgttcgacaacctggagctctatggtgaagctcatgagctgagggacgatccgcccatcattgtcattgaaatctatgaccaggattccatgggcaaagctgacttcatgggccggaccttcgccaaacccctggtgaagatggcagacgaggcgtactgcccaccccgcttcccacctcagctcgagtactaccagatctaccgtggcaacgccacagctggagacctgctggcggccttcgagctgctgcagattggaccagcagggaaggctgacctgccccccatcaatggcccggtggacgtggaccgaggtcccatcatgcccgtgcccatgggcatccggcccgtgctcagcaagtaccgagtggaggtgctgttctggggcctacgggacctaaagcgggtgaacctggcccaggtggaccggccacgggtggacatcgagtgtgcagggaagggggtgcagtcgtccctgatccacaattataagaagaaccccaacttcaacaccctcgtcaagtggtttgaagtggacctcccagagaacgagctgctgcacccgcccttgaacatccgtgtggtggactgccgggccttcggtcgctacacactggtgggctcccatgccgtcagctccctgcgacgcttcatctaccggcccccagaccgctcggcccccagctggaacaccacggtcaggcttctccggcgctgccgtgtgctgtgcaatgggggctcctcctctcactccacaggggaggttgtggtgactatggagccagaggtacccatcaagaaactggagaccatggtgaagctggacgcgacttctgaagctgttgtcaaggtggatgtggctgaggaggagaaggagaagaagaagaagaagaagggcactgcggaggagccagaggaggaggagccagacgagagcatgctggactggtggtccaagtactttgcctccattgacaccatgaaggagcaacttcgacaacaagagccctctggaattgacttggaggagaaggaggaagtggacaataccgagggcctgaaggggtcaatgaagggcaaggagaaggcaagggctgccaaagaggagaagaagaagaaaactcagagctctggctctggccaggggtccgaggcccccgagaagaagaaacccaagattgatgagcttaaggtataccccaaagagctggagtccgagtttgataactttgaggactggctgcacactttcaacttgcttcggggcaagaccggggatgatgaggatggctccaccgaggaggagcgcattgtgggacgcttcaagggctccctctgcgtgtacaaagtgccactcccagaggacgtgtcccgggaagccggctacgactccacctacggcatgttccagggcatcccgagcaatgaccccatcaatgtgctggtccgagtctatgtggtccgggccacggacctgcaccctgctgacatcaacggcaaagctgacccctacatcgccatccggctaggcaagactgacatccgcgacaaggagaactacatctccaagcagctcaaccctgtctttgggaagtcctttgacatcgaggcctccttccccatggaatccatgctgacggtggctgtgtatgactgggacctggtgggcactgatgacctcattggggaaaccaagatcgacctggagaaccgcttctacagcaagcaccgcgccacctgcggcatcgcccagacctactccacacatggctacaatatctggcgggaccccatgaagcccagccagatcctgacccgcctctgcaaagacggcaaagtggacggcccccactttgggccccctgggagagtgaaggtggccaaccgcgtcttcactgggccctctgagattgaggacgagaacggtcagaggaagcccacagacgagcatgtggcgctgttggccctgaggcactgggaggacatcccccgcgcaggctgccgcctggtgccagagcatgtggagacgaggccgctgctcaaccccgacaagccgggcatcgagcagggccgcctggagctgtgggtggacatgttccccatggacatgccagcccctgggacgcctctggacatctcacctcggaagcccaagaagtacgagctgcgggtcatcatctggaacacagatgaggtggtcttggaggacgacgacttcttcacaggggagaagtccagtgacatcttcgtgagggggtggctgaagggccagcaggaggacaagcaggacacagacgtccactaccactccctcactggcgagggcaacttcaactggcgctacctgttccccttcgactacctggcggcggaggagaagatcgtcatctccaagaaggagtccatgttctcctgggacgagaccgagtacaagatccccgcgcggctcaccctgcagatctgggatgcggaccacttctccgctgacgacttcctgggggccatcgagctggacctgaaccggttcccgcggggcgcaaagacagccaagcagtgcaccatggagatggccaccggggaggtggacgtgcccctcgtgtccatcttcaagcaaaagcgcgtcaaaggctggtggcccctcctggcccgcaatgagaacgatgagtttgagctcacgggcaaggtggaggctgagctgcatttactgacagcagaggaggcagagaagaacccagtgggcctggcccgcaatgaacctgaccccctagagaaacccaaccggcccgacacggccttcgtctggttcctcaaccctctcaagtccatcaagtacctcatctgcacccggtacaagtggctcatcatcaagatcgtgctggcgctgttggggctgctcatgttggggctcttcctctacagcctccctggctacatggtcaaaaagctccttggggcatgaaagcttgcc

SEQ ID NO: 9 - DNA, 3822 bp, synthetic construct
  source 1..3822: mol_type = other DNA
cctgcaggcagctgcgcgctcgctcgctcactgaggccgcccgggcaaagcccgggcgtcgggcgacctttggtcgcccggcctcagtgagcgagcgagcgcgcagagagggagtggccaactccatcactaggggttcctgcggccgcacgcgtggagctagcccatatatggagttccggacattgattattgactagttattaatagtaatcaattacggggtcattagttcatagcccatatatggagttccgcgttacataacttacggtaaatggcccgcctggctgaccgcccaacgacccccgcccattgacgtcaataatgacgtatgttcccatagtaacgccaatagggactttccattgacgtcaatgggtggagtatttacggtaaactgcccacttggcagtacatcaagtgtatcatatgccaagtacgccccctattgacgtcaatgacggtaaatggcccgcctggcattatgcccagtacatgaccttatgggactttcctacttggcagtacatctacgtattagtcatcgctattaccatggtgatgcggttttggcagtacatcaatgggcgtggatagcggtttgactcacggggatttccaagtctccaccccattgacgtcaatgggagtttgttttggcaccaaaatcaacgggactttccaaaatgtcgtaacaactccgccccattgacgcaaatgggcggtaggcgtgtacggtgggaggtctatataagcagagctttgggattcgaacatcgattgaattccccggggatcctctaggccaccaagcttgcctcgagccgactgtgccttctagttgccagccatctgttgtttgcccctcccccgtgccttccttgaccctggaaggtgccactcccactgtcctttcctaataaaatgaggaaattgcatcgcattgtctgagtaggtgtcattctattctggggggtggggtggggcaggacagcaagggggaggattgggaagacaatagcaggcatgctggggatgcggtgggctctatggctgattttgtaggtcgacctgctcgagcaggaacccctagtgatggagttggccactccctctctgcgcgctcgctcgctcactgaggccgggcgaccaaaggtcgcccgacgcccgggctttgcccgggcggcctcagtgagcgagcgagcgcgcagctgcctgcaggggcgcctgatgcggtattttctccttacgcatctgtgcggtatttcacaccgcatacgtcaaagcaaccatagtacgcgccctgtagcggcgcattaagcgcggcgggtgtggtggttacgcgcagcgtgaccgctacacttgccagcgccctagcgcccgctcctttcgctttcttcccttcctttctcgccacgttcgccggctttccccgtcaagctctaaatcgggggctccctttagggttccgatttagtgctttacggcacctcgaccccaaaaaacttgatttgggtgatggttcacgtagtgggccatcgccctgatagacggtttttcgccctttgacgttggagtccacgttctttaatagtggactcttgttccaaactggaacaacactcaaccctatctcgggctattcttttgatttataagggattttgccgatttcggcctattggttaaaaaatgagctgatttaacaaaaatttaacgcgaattttaacaaaatattaacgtttacaattttatggtgcactctcagtacaatctgctctgatgccgcatagttaagccagccccgacacccgccaacacccgctgacgcgccctgacgggcttgtctgctcccggcatccgcttacagacaagctgtgaccgtctccgggagctgcatgtgtcagaggttttcaccgtcatcaccgaaacgcgcgagacgaaagggcctcgtgatacgcctatttttataggttaatgtcatgataataatggtttcttagacgtcaggtggcacttttcggggaaatgtgcgcggaacccctatttgtttatttttctaaatacattcaaatatgtatccgctcatgagacaataaccctgataaatgcttcaataatattgaaaaaggaagagtatgagtattcaacatttccgtgtcgcccttattcccttttttgcggcattttgccttcctgtttttgctcacccagaaacgctggtgaaagtaaaagatgctgaagatcagttgggtgcacgagtgggttacatcgaactggatctcaacagcggtaagatccttgagagttttcgccccgaagaacgttttccaatgatgagcacttttaaagttctgctatgtggcgcggtattatcccgtattgacgccgggcaagagcaactcggtcgccgcatacactattctcagaatgacttggttgagtactcaccagtcacagaaaagcatcttacggatggcatgacagtaagagaattatgcagtgctgccataaccatgagtgataacactgcggccaacttacttctgacaacgatcggaggaccgaaggagctaaccgcttttttgcacaacatgggggatcatgtaactcgccttgatcgttgggaaccggagctgaatgaagccataccaaacgacgagcgtgacaccacgatgcctgtagcaatggcaacaacgttgcgcaaactattaactggcgaactacttactctagcttcccggcaacaattaatagactggatggaggcggataaagttgcaggaccacttctgcgctcggcccttccggctggctggtttattgctgataaatctggagccggtgagcgtgggtctcgcggtatcattgcagcactggggccagatggtaagccctcccgtatcgtagttatctacacgacggggagtcaggcaactatggatgaacgaaatagacagatcgctgagataggtgcctcactgattaagcattggtaactgtcagaccaagtttactcatatatactttagattgatttaaaacttcatttttaatttaaaaggatctaggtgaagatcctttttgataatctcatgaccaaaatcccttaacgtgagttttcgttccactgagcgtcagaccccgtagaaaagatcaaaggatcttcttgagatcctttttttctgcgcgtaatctgctgcttgcaaacaaaaaaaccaccgctaccagcggtggtttgtttgccggatcaagagctaccaactctttttccgaaggtaactggcttcagcagagcgcagataccaaatactgtccttctagtgtagccgtagttaggccaccacttcaagaactctgtagcaccgcctacatacctcgctctgctaatcctgttaccagtggctgctgccagtggcgataagtcgtgtcttaccgggttggactcaagacgatagttaccggataaggcgcagcggtcgggctgaacggggggttcgtgcacacagcccagcttggagcgaacgacctacaccgaactgagatacctacagcgtgagctatgagaaagcgccacgcttcccgaagggagaaaggcggacaggtatccggtaagcggcagggtcggaacaggagagcgcacgagggagcttccagggggaaacgcctggtatctttatagtcctgtcgggtttcgccacctctgacttgagcgtcgatttttgtgatgctcgtcaggggggcggagcctatggaaaaacgccagcaacgcggcctttttacggttcctggccttttgctggccttttgctcacatgt